European Patent Application EP 4 410 973 A1, published August 7, 2024. Title: RECOMBINANT YEAST AND APPLICATION THEREOF. Applicant: Shandong Henglu biotech.Co.,Ltd. Application CN PCT/CN2023/077280, filed February 21, 2023. The sequence listing filed with the application follows.

SEQUENCE LISTING (9 sequences)

SEQ ID NO: 1 - protein, 333 aa, Neisseria meningitidis
MQPLVSVLICAYNVEKYFAQSLAAVVNQTWRNLDILIVDDGSTDGTLAIAQRFQEQDGRIRILAQPRNSGLIPSLNIGLDELAKSGGGGEYIARTDADDIAAPDWIEKIVGEMEKDRSIIAMGAWLEVLSEEKDGNRLARHHEHGKIWKKPTRHEDIADFFPFGNPIHNNTMIMRRSVIDGGLRYNTERDWAEDYQFWYDVSKLGRLAYYPEALVKYRLHANQVSSKYSIRQHEIAQGIQKTARNDFLQSMGFKTRFDSLEYRQIKAVAYELLEKHLPEEDFELARRFLYQCFKRTDTLPAGAWLDFAADGRMRRLFTLRQYFGILHRLLKNR

SEQ ID NO: 2 - protein, 398 aa, Helicobacter pylori
MTSASSHSLKEQDFHIPIAFAFDKNYLIAASACIYSLLESIAKANKKIRYTLYALVVGLDEEDEAKLHQIAEPFKEFAALEVKDIEPFLDTIPNPFDEDFTKRFSKMVLVKYFLADLFPQYSKMVWSDVDVIFCNEFSADFLNIKEDDENYFYGVLEVEKHHMMEGFLFCHLDYQRKKNFTLRMHDLLKGNEATEELDFTKWCWPNMKALGIEYCVFPLYYTIKDFSNVYLNENYKKTILEALKNPIIIHYDAWWGAVKPWDYPFGLKADLWLNALSKTPFMSDYTKKMHTNESFYTTKMAQQHYFSSTAPSKEILFKAPYLFFKSYLFVVFKERKIHSRVFELTCGLVKKFFNKLIYFGFFMPKSLAKRVVSKILRVLGLHGIAKKILIKLKLLKKS

SEQ ID NO: 3 - protein, 167 aa, Salmonella enterica
MQPLVSVLICAYNVEKYFAQSLSAVVGQTWRNLDILIVDDGSTDGTPAIARRFQEQDGRIRIISIPRNLGFIASLNIGRDELANRGGGEYIARTDADDIASPGWIEKIVGEMEKDRSIIAMGAWLEVLSEEKDGNRLARHHKHGEIWKKPTRHEDIAAVFPFGNPIH

SEQ ID NO: 4 - protein, 1025 aa, Kluyveromyces lactis
MSCLIPENLRNPKKVHENRLPTRAYYYDQDIFESLNGPWAFALFDAPLDAPDAKNLDWETAKKWSTISVPSHWELQEDWKYGKPIYTNVQYPIPIDIPNPPTVNPTGVYARTFELDSKSIESFEHRLRFEGVDNCYELYVNGQYVGFNKGSRNGAEFDIQKYVSEGENLVVVKVFKWSDSTYIEDQDQWWLSGIYRDVSLLKLPKKAHIEDVRVTTTFVDSQYQDAELSVKVDVQGSSYDHINFTLYEPEDGSKVYDASSLLNEENGNTTFSTKEFISFSTKKNEETAFKINVKAPEHWTAENPTLYKYQLDLIGSDGSVIQSIKHHVGFRQVELKDGNITVNGKDILFRGVNRHDHHPRFGRAVPLDFVVRDLILMKKFNINAVRNSHYPNHPKVYDLFDKLGFWVIDEADLETHGVQEPFNRHTNLEAEYPDTKNKLYDVNAHYLSDNPEYEVAYLDRASQLVLRDVNHPSIIIWSLGNEACYGRNHKAMYKLIKQLDPTRLVHYEGDLNALSADIFSFMYPTFEIMERWRKNHTDENGKFEKPLILCEYGHAMGNGPGSLKEYQELFYKEKFYQGGFIWEWANHGIEFEDVSTADGKLHKAYAYGGDFKEEVHDGVFIMDGLCNSEHNPTPGLVEYKKVIEPVHIKIAHGSVTITNKHDFITTDHLLFIDKDTGKTIDVPSLKPEESVTIPSDTTYVVAVLKDDAGVLKAGHEIAWGQAELPLKVPDFVTETAEKAAKINDGKRYVSVESSGLHFILDKLLGKIESLKVKGKEISSKFEGSSITFWRPPTNNDEPRDFKNWKKYNIDLMKQNIHGVSVEKGSNGSLAVVTVNSRISPVVFYYGFETVQKYTIFANKINLNTSMKLTGEYQPPDFPRVGYEFWLGDSYESFEWLGRGPGESYPDKKESQRFGLYDSKDVEEFVYDYPQENGNHTDTHFLNIKFEGAGKLSIFQKEKPFNFKISDEYGVDEAAHACDVKRYGRHYLRLDHAIHGVGSEACGPAVLDQYRLKAQDFNFEFDLAFE

SEQ ID NO: 5 - protein, 1025 aa, Kluyveromyces marxianus
MSCLIPENLRNPKKVHENRLPTRAYYYDQDIFESLNGPWAFALFDAPLDAPDAKNLDWETAKKWSTISVPSHWELQEDWKYGKPIYTNVQYPIPIDIPNPPTVNPTGVYARTFELDSKSIESFEHRLRFEGVDNCYELYVNGQYVGFNKGSRNGAEFDIQKYVSEGENLVVVKVFKWSDSTYIEDQDQWWLSGIYRDVSLLKLPKKAHIEDVRVTTTFVDSQYQDAELSVKVDVQGSSYDHINFTLYEPEDGSKVYDASSLLNEENGNTTFSTKEFISFSTKKDEETAFKINVKAPEHWTAENPTLYKYQLDLIGSDGSVIQSIKHHVGFRQVELKDGNITVNGKDILFRGVNRHDHHPRFGRAVPLDFVVRDLILMKKFNINAVRNSHYPNHPKVYDLFDKLGFWVIDEADLETHGVQEPFNRHTNLEAEYPDTKNKLYDVNAHYLSDNPEYEVAYLDRASQLVLRDVNHPSIIIWSLGNEACYGRNHKAMYKLIKQLDPTRLVHYEGDLNALSADIFSFMYPTFEIMERWRKNHTDENGKFEKPLILCEYGHAMGNGPGSLKEYQELFYKEKFYQGGFIWEWANHGIEFEDVSTADGKLHKAYAYGGDFKEEVHDGVFIMDGLCNSEHNPTPGLVEYKKVIEPVHIKIAHGSVTITNKHDFITTDHLLFIDKDTGKTIDVPALKPEESVTIPSDTTYVVAVLKDDAGVLKAGHEIAWGQAELPLKVPDFVTETAEKPTKINDGKRYVSVESSGLQFVLDKLLGKIESLKVKGKEISSKFEGSSITFWRPPTNNDEPRDFKNWKKYNIDLMKQNVHEVSVEKGSNGSLAVVTVNSRISPVVFYYGFETVQKYTIFANKINLNTSMKLTGEYQPPDFPRVGYEFWLGDSYESFEWFGRGPGESYPDKKESQRFGLYDSKKVEEFVYDYPQENGNHTDTHFLNIKFEGAGKLSIFQKEKPFNFKISDEYGVDEAAHACDVKRYGRHYLRLDHAIHGVGSEACGPGVLDQYRLKAQDFNFEFDLAFE

SEQ ID NO: 6 - DNA, 534 bp, Kluyveromyces lactis
  source 1..534: mol_type = genomic DNA
tacatatgtatcacgttgacttggtttaaccaggcgacctggtagccagccatacccacacacgttttttgtatcttcagtatagttgtgaaaagtgtagcggaaatttgtggtccgagcaacagcgtctttttctagtagtgcggtcggttacttggttgacattggtatttggactttgttgctacaccattcactacttgaagtcgagtgtgaagggtatgatttctagtggtgaacacctttagttacgtaatgttttcattgctgttttacttgagatttcgattgagaaaaaggtatttaatagctcgaatcaatgtgttatcattgtgaagatgttcttccctaactcgaaaggtatatgaggcttgtgtttcttaggagaattattattcttttgttatgttgcgcttgtagttggaaaaggtgaagagacaaaagcgcttaacacttgaaatttaggaaagagcagaatttggcaaaaaaaataaaaaaaaaataaacacacatactcatcgagaactgaaagat

SEQ ID NO: 7 - DNA, 533 bp, Kluyveromyces marxianus
  source 1..533: mol_type = genomic DNA
tacatatgtatcacgttgacttggtttaaccaggcgacctggtagccagccatacccacacaaacgtttttttgtatattcagtatagttgtgaaaagtgtagcggaaatttgtggtccgagcaacagcgtctttctctagtagcgcggttggttacttggttgatattggcatttggactttgttgctacaccattcactacttgaagtcgagtgtgaagggtatgatttctagtggtgaacaccattagttacgtaatgttttcatcgctgttttacttgagatttcgattgagaaaaaggtatttaatagctcgaatcaatgtgttatcattgtgaaggtgttcttccctaactcgaaaggtatatgaggtttgtgtttcctagtagaattattatccttttcttatgttgcgcttgtagttggaaaaggtgaagagacaaaagcgcttaacacttgaaatttaggaaagagcagaatttggcaaaaaaaaaaaaaaataaacacacatactcatcgagaactgaaagat

SEQ ID NO: 8 - DNA, 188 bp, Saccharomyces cerevisiae
  source 1..188: mol_type = genomic DNA
gcgaatttcttatgatttatgatttttattattaaataagttataaaaaaaataagtgtatacaaattttaaagtgactcttaggttttaaaacgaaaattcttattcttgagtaactctttcctgtaggtcaggttgctttctcaggtatagcatgaggtcgctcttattgaccacacctctaccgg

SEQ ID NO: 9 - DNA, 810 bp, Geneticin
  source 1..810: mol_type = genomic DNA
atgggtaaggaaaagactcacgtttcgaggccgcgattaaattccaacatggatgctgatttatatgggtataaatgggctcgcgataatgtcgggcaatcaggtgcgacaatctatcgattgtatgggaagcccgatgcgccagagttgtttctgaaacatggcaaaggtagcgttgccaatgatgttacagatgagatggtcagactaaactggctgacggaatttatgcctcttccgaccatcaagcattttatccgtactcctgatgatgcatggttactcaccactgcgatccccggcaaaacagcattccaggtattagaagaatatcctgattcaggtgaaaatattgttgatgcgctggcagtgttcctgcgccggttgcattcgattcctgtttgtaattgtccttttaacagcgatcgcgtatttcgtctcgctcaggcgcaatcacgaatgaataacggtttggttgatgcgagtgattttgatgacgagcgtaatggctggcctgttgaacaagtctggaaagaaatgcataagcttttgccattctcaccggattcagtcgtcactcatggtgatttctcacttgataaccttatttttgacgaggggaaattaataggttgtattgatgttggacgagtcggaatcgcagaccgataccaggatcttgccatcctatggaactgcctcggtgagttttctccttcattacagaaacggctttttcaaaaatatggtattgataatcctgatatgaataaattgcagtttcatttgatgctcgatgagtttttctaa